European Patent Specification EP 4 053 273 B1, published September 17, 2025. Title: Novel ferrochelatase variant and a method for producing L-tryptophan using the same. Applicant: CJ CheilJedang Corporation. The sequence listing filed with the application follows.

SEQUENCE LISTING (10 sequences)

SEQ ID NO: 1 - protein, 320 aa, Artificial Sequence
  hemH
MRQTKTGILLANLGTPDAPTPEAVKRYLKQFLSDRRVVDTSRLLWWPLLRGVILPLRSPRVAKLYASVWMEGGSPLMVYSRQQQQALAQRLPEMPVALGMSYGSPSLESAVDELLAEHVDHIVVLPLYPQFSCSTVDAVWDELARILARKRSIPGISFIRDYADNHDYINALANSVRASFAKHGEPDLLLLSYHGIPQRYADEGDDYPQRCRTTTRELASALGMAPEKVMMTFQSRFGREPWLMPYTDETLKMLGEKGVGHIQVMCPGFAADCLETLEEIAEQNREVFLGAGGKKYEYIPALNATPEHIEMMANLVAAYR

SEQ ID NO: 2 - DNA, 963 bp, Artificial Sequence
  hemH
atgcgtcagactaaaaccggtatcctgctggcaaacctgggtacgcccgatgcccccacacctgaagcggtaaaacgctatctgaaacaatttttaagcgacagacgcgtggttgatacctcacggttgttatggtggccattgctgcgcggcgtgattttgccgctgcgctcgccgcgtgtggcgaagctgtatgcctctgtctggatggaaggtggctcgccgctgatggtttacagccgccagcaacagcaggcgctggcacaacgtttaccggagatgcccgtagcgctgggaatgagctacggctcgccatcactggaaagcgccgtagatgaactcctggcagagcatgtagatcatattgtggtgctgccgctttatccgcaattctcctgttctacggtcgatgcggtatgggatgaactggcacgcattctggcgcgcaaacgtagcattccggggatatcgtttatacgtgattacgccgataaccacgattacattaatgcactggcgaacagcgtacgcgcttcttttgccaaacatggcgaaccggatctgctactgctctcttatcatggcattccccagcgttatgcagatgaaggcgatgattacccgcaacgttgccgcacaacgactcgtgaactggcttccgcattggggatggcaccggaaaaagtgatgatgacctttcagtcgcgctttggtcgggaaccctggctgatgccttataccgacgaaacgctgaaaatgctcggagaaaaaggcgtaggtcatattcaggtgatgtgcccgggctttgctgcggattgtctggagacgctggaagagattgccgagcaaaaccgtgaggtcttcctcggtgccggcgggaaaaaatatgaatatattccggcgcttaatgccacgccggaacatatcgaaatgatggctaatcttgttgccgcgtatcgctaa

SEQ ID NO: 3 - protein, 320 aa, Unknown
  hemH
MRQTKTGILLANLGTPDAPTPEAVKRYLKQFLSDRRVVDTSRLLWWPLLRGVILPLRSPRVAKLYASVWMEGGSPLMVYSRQQQQALAQRLPEMPVALGMSYGSPSLESAVDELLAEHVDHIVVLPLYPQFSCSTVGAVWDELARILARKRSIPGISFIRDYADNHDYINALANSVRASFAKHGEPDLLLLSYHGIPQRYADEGDDYPQRCRTTTRELASALGMAPEKVMMTFQSRFGREPWLMPYTDETLKMLGEKGVGHIQVMCPGFAADCLETLEEIAEQNREVFLGAGGKKYEYIPALNATPEHIEMMANLVAAYR

SEQ ID NO: 4 - DNA, 1000 bp, Unknown
  hemH
atgcgtcagactaaaaccggtatcctgctggcaaacctgggtacgcccgatgcccccacacctgaagcggtaaaacgctatctgaaacaatttttaagcgacagacgcgtggttgatacctcacggttgttatggtggccattgctgcgcggcgtgattttgccgctgcgctcgccgcgtgtggcgaagctgtatgcctctgtctggatggaaggtggctcgccgctgatggtttacagccgccagcaacagcaggcgctggcacaacgtttaccggagatgcccgtagcgctgggaatgagctacggctcgccatcactggaaagcgccgtagatgaactcctggcagagcatgtagatcatattgtggtgctgccgctttatccgcaattctcctgttctacggtcggtgcggtatgggatgaactggcacgcattctggcgcgcaaacgtagcattccggggatatcgtttatacgtgattacgccgataaccacgattacattaatgcactggcgaacagcgtacgcgcttcttttgccaaacatggcgaaccggatctgctactgctctcttatcatggcattccccagcgttatgcagatgaaggcgatgattacccgcaacgttgccgcacaacgactcgtgaactggcttccgcattggggatggcaccggaaaaagtgatgatgacctttcagtcgcgctttggtcgggaaccctggctgatgccttataccgacgaaacgctgaaaatgctcggagaaaaaggcgtaggtcatattcaggtgatgtgcccgggctttgctgcggattgtctggagacgctggaagagattgccgagcaaaaccgtgaggtcttcctcggtgccggcgggaaaaaatatgaatatattccggcgcttaatgccacgccggaacatatcgaaatgatggctaatcttgttgccgcgtatcgctaaagctgagcggtaaagaactgagcgccgtcgcgaagag

SEQ ID NO: 5 - DNA, 40 bp, Artificial Sequence
  Forward Primer
ggaattcgagctcggtacccatgcgtcagactaaaaccgg

SEQ ID NO: 6 - DNA, 21 bp, Artificial Sequence
  Reverse Primer
cataccgcatcgaccgtagaa

SEQ ID NO: 7 - DNA, 21 bp, Artificial Sequence
  Forward Primer
ttctacggtcgatgcggtatg

SEQ ID NO: 8 - DNA, 40 bp, Artificial Sequence
  Reverse Primer
gttatccctagcggatccccttagcgatacgcggcaacaa

SEQ ID NO: 9 - DNA, 21 bp, Artificial Sequence
  Forward Primer
gacctctcacagcaattagtt

SEQ ID NO: 10 - DNA, 20 bp, Artificial Sequence
  Reverse Primer
cgacgaggctcttcgcgacg